European Patent Specification EP 3 843 775 B1, published April 3, 2024. Title: METHODS OF TREATING AN AUTOIMMUNE DISEASE. Applicant: THE GOVERNING COUNCIL OF THE UNIVERSITY OF TORONTO. Application PCT/CA2019/051200. The sequence listing filed with the application follows.

SEQUENCE LISTING (4 sequences)

SEQ ID NO: 1 - protein, 285 aa, Homo sapiens
MDDSTEREQSRLTSCLKKREEMKLKECVSILPRKESPSVRSSKDGKLLAATLLLALLSCCLTVVSFYQVAALQGDLASLRAELQGHHAEKLPAGAGAPKAGLEEAPAVTAGLKIFEPPAPGEGNSSQNSRNKRAVQGPEETVTQDCLQLIADSETPTIQKGSYTFVPWLLSFKRGSALEEKENKILVKETGYFFIYGQVLYTDKTYAMGHLIQRKKVHVFGDELSLVTLFRCIQNMPETLPNNSCYSAGIAKLEEGDELQLAIPRENAQISLDGDVTFFGALKLL

SEQ ID NO: 2 - DNA, 2665 bp, Homo sapiens
gaaattcttacaaaaactgaaagtgaaatgaggaagacagattgagcaatccaatcggagggtaaatgccagcaaacctactgtacagtaggggtagagatgcagaaaggcagaaaggagaaaattcaggataactctcctgaggggtgagccaagccctgccatgtagtgcacgcaggacatcaacaaacacagataacaggaaatgatccattccctgtggtcacttattctaaaggccccaaccttcaaagttcaagtagtgatatggatgactccacagaaagggagcagtcacgccttacttcttgccttaagaaaagagaagaaatgaaactgaaggagtgtgtttccatcctcccacggaaggaaagcccctctgtccgatcctccaaagacggaaagctgctggctgcaaccttgctgctggcactgctgtcttgctgcctcacggtggtgtctttctaccaggtggccgccctgcaaggggacctggccagcctccgggcagagctgcagggccaccacgcggagaagctgccagcaggagcaggagcccccaaggccggcctggaggaagctccagctgtcaccgcgggactgaaaatctttgaaccaccagctccaggagaaggcaactccagtcagaacagcagaaataagcgtgccgttcagggtccagaagaaacagtcactcaagactgcttgcaactgattgcagacagtgaaacaccaactatacaaaaaggatcttacacatttgttccatggcttctcagctttaaaaggggaagtgccctagaagaaaaagagaataaaatattggtcaaagaaactggttacttttttatatatggtcaggttttatatactgataagacctacgccatgggacatctaattcagaggaagaaggtccatgtctttggggatgaattgagtctggtgactttgtttcgatgtattcaaaatatgcctgaaacactacccaataattcctgctattcagctggcattgcaaaactggaagaaggagatgaactccaacttgcaataccaagagaaaatgcacaaatatcactggatggagatgtcacattttttggtgcattgaaactgctgtgacctacttacaccatgtctgtagctattttcctccctttctctgtacctctaagaagaaagaatctaactgaaaataccaaaaaaaaaaaaaaaaaaaaagtagttaccattgccttttctgtgagctatttgttttggtttgctgaaactagtccaaaacaggaaatttaacagacagccacagccaaagagtgtcatgtgaattacaagaaatagagcccatttagggaaagatagaactagaaaggcttttcattataattccatgttgaacaattgagtcatagcttcttatcttggaggaaggacacaattcaaaggggcagtaaggattttgtaaaacgtggcatccataatttactatggagcaagtgcccacatctctaggacattaagacatttatgagaaatctcaggattcatcttctgtttttatgttaaatgcactccctccttttcagttaacattataaaaagtaaaaaatgaaaattttagaaatcttgcattagacacatgaaaaaataactaaaagtttaaatttaaatatgaaacaattttgctgaaaatagtatccatatactatttaagtcttttatggttatttcaagtatacaatttctatctgtaatgtaatatattacccacacatttttttcacaggagagagagaatatcctcatttgtttatgctcatgtgtattttctatagtgaatttcagaaacttttaatatcaggtaatttcaatttatgcctataaagcattgattgaaaaataactagaattgtgcatatataacacataatctccaacagaagttactgaatacattcatactaatgtaatgtaatttccctttatttcttgctcttctgtttcaaactgctgctattgtagtttacatatcccaacctttaaaaatattcctcttattagctttatattcactttatagaagttgagttttaattaaaattcttggcatcctgaagtatgtcacatagcatgtgctccttataaatatgttgatatctcagaagacagcatcccggttttcattttataaagtaccatacttaagaatgctgtaatacttatcttttataacatgtttccttcgctttgcttgtcttttatgtcatcagttttaactgtttacttcatttaacagtttacatcattcaacagtttacttcattaaacagtaggtggaaaaatagatgccagtctatgaaaatcttcccatctatatcaaaatacttttcaaggatatacttttcaaaacaaacgatttaaattttatgtttaaaatataaactttagatttaaactttatttaaatatctggttcctatgattttgacttcagtaagttcaaataaaatatattttgcaattcatttttacattataatttaaaaagaagaagcgataagtggagtcagtttcaatgctaggtggggtggttaatgatttttctggtgttgctgctaatgtggattaacaaataaaaacattcattgccttttgcctcataaaa

SEQ ID NO: 3 - protein, 309 aa, Mus musculus
MDESAKTLPPPCLCFCSEKGEDMKVGYDPITPQKEEGAWFGICRDGRLLAATLLLALLSSSFTAMSLYQLAALQADLMNLRMELQSYRGSATPAAAGAPELTAGVKLLTPAAPRPHNSSRGHRNRRAFQGPEETEQDVDLSAPPAPCLPGCRHSQHDDNGMNLRNIIQDCLQLIADSDTPTIRKGTYTFVPWLLSFKRGNALEEKENKIVVRQTGYFFIYSQVLYTDPIFAMGHVIQRKKVHVFGDELSLVTLFRCIQNMPKTLPNNSCYSAGIARLEEGDEIQLAIPRENAQISRNGDDTFFGALKLL

SEQ ID NO: 4 - DNA, 1699 bp, Mus musculus
aggcagattgagcaatccatggaaggccagagccagagaacctacttcagggtagcaaaagatgcagaagaaagtcaggagagcgctcctgggggaacccagccctgccatgctctgagggcagtctcccaggacacagatgacaggaaatgacccacccctgtggtcacttactccaaaggcctagaccttcaaagtgctcctcgtggaatggatgagtctgcaaagaccctgccaccaccgtgcctctgtttttgctccgagaaaggagaagatatgaaagtgggatatgatcccatcactccgcagaaggaggagggtgcctggtttgggatctgcagggatggaaggctgctggctgctaccctcctgctggccctgttgtccagcagtttcacagcgatgtccttgtaccagttggctgccttgcaagcagacctgatgaacctgcgcatggagctgcagagctaccgaggttcagcaacaccagccgccgcgggtgctccagagttgaccgctggagtcaaactcctgacaccggcagctcctcgaccccacaactccagccgcggccacaggaacagacgcgctttccagggaccagaggaaacagaacaagatgtagacctctcagctcctcctgcaccatgcctgcctggatgccgccattctcaacatgatgataatggaatgaacctcagaaacatcattcaagactgtctgcagctgattgcagacagcgacacgccgactatacgaaaaggaacttacacatttgttccatggcttctcagctttaaaagaggaaatgccttggaggagaaagagaacaaaatagtggtgaggcaaacaggctatttcttcatctacagccaggttctatacacggaccccatctttgctatgggtcatgtcatccagaggaagaaagtacacgtctttggggacgagctgagcctggtgaccctgttccgatgtattcagaatatgcccaaaacactgcccaacaattcctgctactcggctggcatcgcgaggctggaagaaggagatgagattcagcttgcaattcctcgggagaatgcacagatttcacgcaacggagacgacaccttctttggtgccctaaaactgctgtaactcacttgctggagtgcgtgatccccttccctcgtcttctctgtacctccgagggagaaacagacgactggaaaaactaaaagatggggaaagccgtcagcgaaagttttctcgtgacccgttgaatctgatccaaaccaggaaatataacagacagccacaaccgaagtgtgccatgtgagttatgagaaacggagcccgcgctcagaaagaccggatgaggaagaccgttttctccagtcctttgccaacacgcaccgcaaccttgctttttgccttgggtgacacatgttcagaatgcagggagatttccttgttttgcgatttgccatgagaagagggcccacaactgcaggtcactgaagcattcacgctaagtctcaggatttactctcccttctcatgctaagtacacacacgctcttttccaggtaatactatgggatactatggaaaggttgtttgtttttaaatctagaagtcttgaactggcaatagacaaaaatccttataaattcaagtgtaaaataaacttaattaaaaaggtttaagtgtgaaa